European Patent Application EP 4 321 174 A1, published February 14, 2024. Title: NOVEL TARGET FOR ANTI-CANCER AND IMMUNE-ENHANCING. Applicant: Genome and Company. The sequence listing filed with the application follows.

SEQUENCE LISTING (13 sequences)

SEQ ID NO: 1 - RNA, 21 nt, Artificial Sequence
  human CNTN4 siRNA_sense
caguaucuuugccagaagutt

SEQ ID NO: 2 - RNA, 21 nt, Artificial Sequence
  human CNTN4 siRNA_antisense
acuucuggcaaagauacugtt

SEQ ID NO: 3 - RNA, 21 nt, Artificial Sequence
  human CNTN4 siRNA_sense
gauaaugagucggaaguaatt

SEQ ID NO: 4 - RNA, 21 nt, Artificial Sequence
  human CNTN4 siRNA_antisense
uuacuuccgacucauuauctt

SEQ ID NO: 5 - RNA, 21 nt, Artificial Sequence
  human CNTN4 siRNA_sense
gugacaauagacgaaaucatt

SEQ ID NO: 6 - RNA, 21 nt, Artificial Sequence
  human CNTN4 siRNA_antisense
ugauuucgucuauugucactt

SEQ ID NO: 7 - RNA, 19 nt, Artificial Sequence
  mouse CNTN4 siRNA_sense
guguagacaaacucucugu

SEQ ID NO: 8 - RNA, 19 nt, Artificial Sequence
  mouse CNTN4 siRNA_antisense
acagagaguuugucuacac

SEQ ID NO: 9 - protein, 201 aa, Artificial Sequence
  FN1 ~ FN2 domain
PPEAVTIDEITDTTAQLSWRPGPDNHSPITMYVIQARTPFSVGWQAVSTVPELIDGKTFTATVVGLNPWVEYEFRTVAANVIGIGEPSRPSEKRRTEEALPEVTPANVSGGGGSKSELVITWETVPEELQNGRGFGYVVAFRPYGKMIWMLTVLASADASRYVFRNESVHPFSPFEVKVGVFNNKGEGPFSPTTVVYSAEE

SEQ ID NO: 10 - protein, 15 aa, Artificial Sequence
  KPI domain
RAMISRWYFDVTEGK

SEQ ID NO: 11 - protein, 102 aa, Artificial Sequence
  scFv AB1 VL
ALTQPSSVSANLGETVKITCSGSSGSYGWYQQKSPGSAPVTLIYDNTNRPSDIPSRFSGSGSGSTGTLTITGVRAEDEAVYYCGGYDGSTDVFGAGTTLTVL

SEQ ID NO: 12 - protein, 123 aa, Artificial Sequence
  scFv AB1 VH
AVTLDESEGGLQTPGGALSLVCKASGFTFSSFNMFWVRQAPGKGLEYVAEISGGGGSTWYAPAVKGRATISRDNGQSTVRLQLNNLRAEDTGTYYCAKSADTWSYGAATIDAWGHGTEVIVSS

SEQ ID NO: 13 - protein, 98 aa, Artificial Sequence
  Domain 8 (FN2 Domain)
TPANVSGGGGSKSELVITWETVPEELQNGRGFGYVVAFRPYGKMIWMLTVLASADASRYVFRNESVHPFSPFEVKVGVFNNKGEGPFSPTTVVYSAEE